European Patent Application EP 4 261 209 A1, published October 18, 2023. Title: Method for nucleic acid detection, compounds, and fluorescent probe. Applicant: Wakayama University. The sequence listing filed with the application follows.

SEQUENCE LISTING (6 sequences)

SEQ ID NO: 1 - DNA, 14 bp, Unknown
  Double-stranded DNA
  Inventor: Sakamoto, Takashi
gcgcaaatttgcgc

SEQ ID NO: 2 - DNA, 14 bp, Unknown
  Double-stranded DNA
gcgcaagcttgcgc

SEQ ID NO: 3 - DNA, 27 bp, Quadruplex DNA
ttagggttagggttagggttagggtta

SEQ ID NO: 4 - DNA, 26 bp, Unknown
  Quadruplex DNA
aaagggttagggttagggttagggaa

SEQ ID NO: 5 - DNA, 22 bp, Unknown
  Quadruplex DNA
tgagggtgggtagggtgggtaa

SEQ ID NO: 6 - DNA, 12 bp, Unknown
  Double-stranded DNA
cttttgcaaaag